European Patent Specification EP 3 169 778 B1, published October 25, 2023. Title: NANOS KNOCKOUT THAT ABLATES GERMLINE CELLS. Applicant: Washington State University University of Maryland The University of Edinburgh. The sequence listing filed with the application follows.

SEQUENCE LISTING (204 sequences)

SEQ ID NO: 1 - DNA, 417 bp, Sus scrofa
atgcagctgccaccctttgacatgtggaaggactacttcaacctgagccaggtggtgttgggactgatccagaatcgtcgacaagggccagaggccccgggcaccggggagccaagacctgagcccccactggagcaggaccagggcccgggagagcggggggccagcggggggctggccaccctgtgcaacttttgcaaacacaatggggaatctcgccacgtgtactcctcgcaccagctgaagacaccggagggcgtggtggtgtgtcccatcctacgacactatgtgtgtcccctgtgcggggccaccggtgaccaggctcacacactcaagtactgcccgctcaacggcggccagcagtctctctatcgccgcagtgggcgcaattcagccggccgcaaggtcaagcgctga

SEQ ID NO: 2 - protein, 138 aa, Sus scrofa
MQLPPFDMWKDYFNLSQVVLGLIQNRRQGPEAPGTGEPRPEPPLEQDQGPGERGASGGLATLCNFCKHNGESRHVYSSHQLKTPEGVVVCPILRHYVCPLCGATGDQAHTLKYCPLNGGQQSLYRRSGRNSAGRKVKR

SEQ ID NO: 3 - DNA, 1073 bp, Sus scrofa
cagcccacccagggaccatgcattcctttggcaggtgcatttttggaggagcagcagcaagcccccctgtgacaataaggaacctcccacagcctgctcctccctcttcacacccccttggaggtataaggagggaactgacagcccagactcctgggctccagagagagaaagggaggggcagggggaaggggatagaaggacgatctttggggtggctgggtttcttctctctctctgccctttcacctggtacactttgcccagccatggggaccttcaacctgtggacagattacctgggtttggcacgcctggtgggggctctgcgtggggaagaggaacctgagacgaggctggacccccagccagcaccagtgccaggaccagagggtcagaggcccagcccggaatcctcaccagctcctgaacgcctgtgctctttctgcaaacataatggcgaatcccgggccatctaccagtcccacgtgctcaaggatgaagcgggccgagttctgtgccccattcttcgagactacgtgtgcccccagtgcggtgccacacgcgagcgtgcccatacccgccgcttctgccctctcaccagccagggctacacctctgtctacagctacaccacccgcaactcggccggcaagaagctggcccgcccggacaaggcgaggacacaggactctggacatcggcgaggaggaggaggaggaggtgccagcacaggttccaaaggtgccgggaagtcttctggaacttctccgtctccctgctgtccctccacttctgcctaagaggctggcgcgagcaggacggagatgctgccttcacctggggatggggacccaggctcagtggaggctgggtttcagggacgacctacccttcgcggatccgcccctgcccccagcctgggagccctgcaagggagccaggcctggaagctcggccaaaagagagccgctcctttctccccatctcccaccccaagaaaggaggtggtcctctggcaaccctgccctccttccccagcgctgggcacccagttagcactcaataaatac

SEQ ID NO: 4 - protein, 261 aa, Sus scrofa
MHSFGRCIFGGAAASPPVTIRNLPQPAPPSSHPLGGIRRELTAQTPGLQREKGRGRGKGIEGRSLGWLGFFSLSALSPGTLCPAMGTFNLWTDYLGLARLVGALRGEEEPETRLDPQPAPVPGPEGQRPSPESSPAPERLCSFCKHNGESRAIYQSHVLKDEAGRVLCPILRDYVCPQCGATRERAHTRRFCPLTSQGYTSVYSYTTRNSAGKKLARPDKARTQDSGHRRGGGGGGASTGSKGAGKSSGTSPSPCCPSTSA

SEQ ID NO: 5 - DNA, 1906 bp, Sus scrofa
cgcagggggcagggccgcggcagcgaggccggggggcggggaggagcggggcccgataaaaggcagcgaggcggccccaccccgctgcaggccggcgggcaggctcggcgcgtcctttccgtccggcccgcgccggcggcggggaggcggcgcgcgcggcccgcagcccgcccatggaggctttcccctgggcgccccgctcgccccgccgcggccgcgtccccccgcccatggcgctcgtgcccagcgcccgctacgtgagcgcccagggcccggcgcacccgcaacccttcagctcgtggaacgactacctgggactcgccacgctcatcaccaaggcggtggacggcgagccgcgctttggctgcgcccgcggcgaggacggcggcggcggcggcggctccccaccctcctcttcctcctcgtcgtgctgctccccccacgcgggggccgggcctggggcgctggggcccgcgctggggccacccgactacgacgaggacgacgacgacgacagcgacgagccggggtcccggggccgctacctggggggcacgctggagctgcgcgcgctggagctgtgcgcggacccctcggaggccgggctgctggaggagcgcttcgccgagctgagcccgttcgcgggtcgcgccaccgctgtgctgctgggctgggcacccgccactgccgccaccgccgaggcggcaccgcgcgaggagcgggccccggcgtgggcggccgagccccggctgcacgcagcctttggggcggccggcgcccggctgctcaagcccgagctgcaggtgtgtgtgttttgccggaacaacaaggaggcggtggcgctctacaccacccacatcttgaagggacccgacgggcgagtgctgtgccccgtgctgcgccgctacacgtgtcccctgtgcggcgccagcggcgacaacgcgcacaccatcaagtactgcccgctctccaaagtgccgccgccgcgcagcgtcagggacggcctgcccggcaagaagctgcgctgagggcccggactccggtctgctactgccacctgacgccaccagggtcgccgcctgcccaatgtctagtttggcctgcgcaccatctctctctctcgctgctgaggagcgtggagctcagctgttggttgaacttgagatgtactgattttttttttttttttttcaaaagaacccggcggtactgagtcctttcctgtcgaagagcgcttaagactagaagctaaaatcttgatttgtttatctctagtttgtgcacatccagacggtgaaggctgggtgttcgttccactaactgaaatgtggcaacttagaagtgtttatttactctatacgtcaacctattttagatgcgcatcagtatatgaaattgtctcaatctaatcttggatgtttaattttatgaatggaggcactttactaggcctagaatatttttttaaaagcctctaaactgaacttaactggcgattttatggaatgtcagcaaaatgacttttattgtttgaaacaagtaataatatttctgttgtccttaatcagttattctaattccaggtgaagcaaccctcacctgcctggtagcatcattaagtgaaggcttagtaaactttccagtgttagtttgggtgggtgttccccccgtggcttgtttctgtcctagctggaggtgtaaagatgtacaatctgtggcaggtagaatacagctccttatccttttatgtaccacatcttttattactgaacgagcaactagcgtttcccatctttcaaagtcgtgccaggttatataatattgtgtatacacttggaaatggtgctgtttaaaagaatttgtgtatttatacagtaacagtatatgaattcattaatcttgtctt

SEQ ID NO: 6 - protein, 284 aa, Sus scrofa
MEAFPWAPRSPRRGRVPPPMALVPSARYVSAQGPAHPQPFSSWNDYLGLATLITKAVDGEPRFGCARGEDGGGGGGSPPSSSSSSCCSPHAGAGPGALGPALGPPDYDEDDDDDSDEPGSRGRYLGGTLELRALELCADPSEAGLLEERFAELSPFAGRATAVLLGWAPATAATAEAAPREERAPAWAAEPRLHAAFGAAGARLLKPELQVCVFCRNNKEAVALYTTHILKGPDGRVLCPVLRRYTCPLCGASGDNAHTIKYCPLSKVPPPRSVRDGLPGKKLR

SEQ ID NO: 7 - DNA, 23 bp, Sus scrofa
gaagacaccggagggcgtggtgg

SEQ ID NO: 8 - DNA, 23 bp, Sus scrofa
gaatcgtcgacaagggccagagg

SEQ ID NO: 9 - DNA, 548 bp, Bovine
tcagctgctcctgtctgcgggcccccagcccacttctctccagccacccaccaccaacactcccccgggtgccatgcagctgccaccctttgacatgtggaaggactacttcaacctgagccaagtggtgctggcactgatccagagtcgggggcaagggttggagacccaagggactggggagccgagacccgggccccatgtggagcaggatcaggggcagggcggacgcggggctggcgggggcctggccaccctgtgcaacttttgcaaacacaatggagagtctcgccacgtgtactcctcacaccagctgaagaccccggagggcgtggtggtgtgtcccattctgcggcattatgtatgtcccctgtgcggggccaccggggaccaggcccacacactcaagtactgcccactcaacggaggacagcagtctctctaccgccgcagtgggcgcaactcagccggccgcaaggtcaagcgctgaagaccgtcaggtacccacccgctgcagccccaaccctccctggttcagccctcccaag

SEQ ID NO: 10 - protein, 138 aa, Bovine
MQLPPFDMWKDYFNLSQVVLALIQSRGQGLETQGTGEPRPGPHVEQDQGQGGRGAGGGLATLCNFCKHNGESRHVYSSHQLKTPEGVVVCPILRHYVCPLCGATGDQAHTLKYCPLNGGQQSLYRRSGRNSAGRKVKR

SEQ ID NO: 11 - DNA, 1624 bp, Bovine
gccgccgccgcggccaccgccgaagcagcaccgcgagaggagcgggccccggcgtgggcggccgagcccaagctgcacgccgcctccggggcggccgccgcccggctgctcaagcccgagctgcaggtgtgcgtgttttgccggaacaacaaggaggcggtggcgctctacaccacccacatcctgaagggacccgacgggcgggtgctgtgccccgtgctgcgccggtacacgtgtcccctgtgcggtgccagcggcgacaacgcgcacaccatcaagtactgcccgctttccaaagtgccgccgccgcctgcagcccgcccgccgccgcgcagcgcccgggacggcctgcccggcaagaagctgcgctaagggcccggaccccggtctgctgctgccacctgatgccactggggtagccgcccgcccactctcgtgtttggtctgcgcaccatctcttcctcgctgccggggagtgtggagctcgtcttggtttttccagaggaagccgacggtaccgagtattttcctaacgaagagcagttgagactagacgttaaaattttgattaatgtttctagtttgtgcacatccagatggtgaaggctgggtattccactaactgaaatgtggcaacttagaggcgctgtggtttatttatacgtcgacctattttagatgcgcatcagtatgaaattgtctcagtctaatcttggatgtttaattttatgaatggaggcactttactaggtctagaatatttttttaaaagcctctcaactgaacttaaaactggcgattttatggagtgtcagcaaaatgactattttattgtctgaaacaatatttctgttgtccttacccagttgtaattccaggtgaagccctgcgtggtagcatcattaagtgaagacttggtatgctttacagtgttagtttgggtgggtgttccctccttgtggcttgtttttgtcctagctggagatgtataaaatgtacaatttgtaggtagcaggtagaatacagctcatgtaccagatctttttattactgaacgagcaactactaccgtttttcccctttaaaaatagtgccaagttataatcatattgtgtatacacttgaaaatggtgctgtttaaaaaaattgtgtatttatacagtaacagtatatgaattcattaaccttgcctttaactctacttggctttttctttatgccccttcctattccagttcttcaaaaatatgtgatacttaagatcaaacgggtgcaataactcattcactctgaattgctccatttcagggtctctaaatagtggaaatctcattccagctgttgcctctcagactaaatgtaagatggaatcctttgagctctggaaggttaatgaaacaactggtgttcaggaaggttccactctggactgtgtcagctttaaaccatcacagaagtcctcaaaccagtataagtaccaattaaaggaactgactgggtgtagggggggtaacacaaggaacacagcctccatctattgtgttcccattctcattagaagacaacccttctggaatcccaccagttattttcatcggtgagattaaatctaatcttgggcaaa

SEQ ID NO: 12 - protein, 123 aa, Bovine
AAAAATAEAAPREERAPAWAAEPKLHAASGAAAARLLKPELQVCVFCRNNKEAVALYTTHILKGPDGRVLCPVLRRYTCPLCGASGDNAHTIKYCPLSKVPPPPAARPPPRSARDGLPGKKLR

SEQ ID NO: 13 - DNA, 2056 bp, Bovine
cgctacgtgagcacccagggcccggcgcacccgcagcccttcagctcgtggaacgactatctgggactcgccacgctcatcaccaaggcggtggacggcgagccgcgcttcggctgcgcccgcggcggggacggcggcggggacggctccccgccttcttcttcctcctcgtcgtgctgctccccccacgtgggggccgggcctggggcgctggggcccgcgctggggccgcccgactacgacgaggacgacgacgacgacgacagcgacgatccggggtcccggagccgctacctggggggcgcgctggagctgcgcgcgctggagctgtgcgcggaccctgccgaggccgggctgctggaggagcgtttcgctgagctgagcccgttcgctggtcgcgccgctgccgtgcttctgggctgcgcacccgccgccgccgccgcggccaccgccgaagcagcaccgcgagaggagcgggccccggcgtgggcggccgagcccaagctgcacgccgcctccggggcggccgccgcccggctgctcaagcccgagctgcaggtgtgcgtgttttgccggaacaacaaggaggcggtggcgctctacaccacccacatcctgaagggacccgacgggcgggtgctgtgccccgtgctgcgccggtacacgtgtcccctgtgcggtgccagcggcgacaacgcgcacaccatcaagtactgcccgctttccaaagtgccgccgccgcctgcagcccgcccgccgccgcgcagcgcccgggacggcctgcccggcaagaagctgcgctaagggcccggaccccggtctgctgctgccacctgatgccactggggtagccgcccgcccactctcgtgtttggtctgcgcaccatctcttcctcgctgccggggagtgtggagctcgtcttggtttttccagaggaagccgacggtaccgagtattttcctaacgaagagcagttgagactagacgttaaaattttgattaatgtttctagtttgtgcacatccagatggtgaaggctgggtattccactaactgaaatgtggcaacttagaggcgctgtggtttatttatacgtcgacctattttagatgcgcatcagtatgaaattgtctcagtctaatcttggatgtttaattttatgaatggaggcactttactaggtctagaatatttttttaaaagcctctcaactgaacttaaaactggcgattttatggagtgtcagcaaaatgactattttattgtctgaaacaatatttctgttgtccttacccagttgtaattccaggtgaagccctgcgtggtagcatcattaagtgaagacttggtatgctttacagtgttagtttgggtgggtgttccctccttgtggcttgtttttgtcctagctggagatgtataaaatgtacaatttgtaggtagcaggtagaatacagctcatgtaccagatctttttattactgaacgagcaactactaccgtttttcccctttaaaaatagtgccaagttataatcatattgtgtatacacttgaaaatggtgctgtttaaaaaaattgtgtatttatacagtaacagtatatgaattcattaaccttgcctttaactctacttggctttttctttatgccccttcctattccagttcttcaaaaatatgtgatacttaagatcaaacgggtgcaataactcattcactctgaattgctccatttcagggtctctaaatagtggaaatctcattccagctgttgcctctcagactaaatgtaagatggaatcctttgagctctggaaggttaatgaaacaactggtgttcaggaaggttccactctggactgtgtcagctttaaaccatcacagaagtcctcaaaccagtataagtaccaattaaaggaactgactgggtgtagggggggtaacacaaggaacacagcctccatctattgtgttcccattctcattagaagacaacccttctggaatcccaccagttattttcatcggtgagattaaatctaatcttgggcaaa

SEQ ID NO: 14 - protein, 267 aa, Bovine
RYVSTQGPAHPQPFSSWNDYLGLATLITKAVDGEPRFGCARGGDGGGDGSPPSSSSSSCCSPHVGAGPGALGPALGPPDYDEDDDDDDSDDPGSRSRYLGGALELRALELCADPAEAGLLEERFAELSPFAGRAAAVLLGCAPAAAAAATAEAAPREERAPAWAAEPKLHAASGAAAARLLKPELQVCVFCRNNKEAVALYTTHILKGPDGRVLCPVLRRYTCPLCGASGDNAHTIKYCPLSKVPPPPAARPPPRSARDGLPGKKLR

SEQ ID NO: 15 - DNA, 482 bp, Artificial Sequence
  Synthetic polynucleotide
agttaactaagctttgtacaaaaaagcaggctttaaaggaaccaattcagtcgactggatccggtaccaaggtcgggcaggaagagggcctatttcccatgattccttcatatttgcatatacgatacaaggctgttagagagataattagaattaatttgactgtaaacacaaagatattagtacaaaatacgtgacgtagaaagtaataatttcttgggtagtttgcagttttaaaattatgttttaaaatggactatcatatgcttaccgtaacttgaaagtatttcgatttcttggctttatatatcttgtggaaaggacgaaacaccgaatcgtcgacaagggccaggttttagagctagaaatagcaagttaaaataaggctagtccgttatcaacttgaaaaagtggcaccgagtcggtgctttttttctagacccagctttcttgtacaaagttggcattactcgagatccact

SEQ ID NO: 16 - DNA, 482 bp, Artificial Sequence; identical to SEQ ID NO: 15
  Synthetic polynucleotide

SEQ ID NO: 17 - DNA, 482 bp, Artificial Sequence
  Synthetic polynucleotide
agttaactaagctttgtacaaaaaagcaggctttaaaggaaccaattcagtcgactggatccggtaccaaggtcgggcaggaagagggcctatttcccatgattccttcatatttgcatatacgatacaaggctgttagagagataattagaattaatttgactgtaaacacaaagatattagtacaaaatacgtgacgtagaaagtaataatttcttgggtagtttgcagttttaaaattatgttttaaaatggactatcatatgcttaccgtaacttgaaagtatttcgatttcttggctttatatatcttgtggaaaggacgaaacaccgtggcccttgtcgacgattcgttttagagctagaaatagcaagttaaaataaggctagtccgttatcaacttgaaaaagtggcaccgagtcggtgctttttttctagacccagctttcttgtacaaagttggcattactcgagatccact

SEQ ID NO: 18 - DNA, 318 bp, Artificial Sequence
  Synthetic polynucleotide
tgtacaaaaaagcaggctttaaaggaaccaattcagtcgactggatccggtaccaaggtcgggcaggaagagggcctatttcccatgattccttcatatttgcatatacgatacaaggctgttagagagataattagaattaatttgactgtaaacacaaagatattagtacaaaatacgtgacgtagaaagtaataatttcttgggtagtttgcagttttaaaattatgttttaaaatggactatcatatgcttaccgtaacttgaaagtatttcgatttcttggctttatatatcttgtggaaaggacgaaacacc

SEQ ID NO: 19 - DNA, 20 bp, Artificial Sequence
  Synthetic oligonucleotide
gtggcccttgtcgacgattc

SEQ ID NO: 20 - DNA, 76 bp, Artificial Sequence
  Synthetic polynucleotide
gttttagagctagaaatagcaagttaaaataaggctagtccgttatcaacttgaaaaagtggcaccgagtcggtgc

SEQ ID NO: 21 - DNA, 10 bp, Artificial Sequence
  Synthetic oligonucleotide
  misc_feature (8)..(10): n is a, c, g, or t
tttttttnnn

SEQ ID NO: 22 - DNA, 360 bp, Artificial Sequence
  Synthetic polynucleotide
gagggcctatttcccatgattccttcatatttgcatatacgatacaaggctgttagagagataattggaattaatttgactgtaaacacaaagatattagtacaaaatacgtgacgtagaaagtaataatttcttgggtagtttgcagttttaaaattatgttttaaaatggactatcatatgcttaccgtaacttgaaagtatttcgatttcttggctttatatatcttgtggaaaggacgaaacaccgggtcttcgagaagacctgttttagagctagaaatagcaagttaaaataaggctagtccgttatcaacttgaaaaagtggcaccgagtcggtgcttttttgttttagagct

SEQ ID NO: 23 - DNA, 240 bp, Artificial Sequence
  Synthetic oligonucleotide
tttcccatgattccttcatatttgcatatacgatacaaggctgttagagagataattggaattaatttgactgtaaacacaaagatattagtacaaaatacgtgacgtagaaagtaataatttcttgggtagtttgcagttttaaaattatgttttaaaatggactatcatatgcttaccgtaacttgaaagtatttcgatttcttggctttatatatcttgtggaaaggacgaaacacc

SEQ ID NO: 24 - DNA, 76 bp, Artificial Sequence; identical to SEQ ID NO: 20
  Synthetic oligonucleotide

SEQ ID NO: 25 - DNA, 10 bp, Artificial Sequence
  Synthetic oligonucleotide
  misc_feature (7)..(10): n is a, c, g, or t
ttttttnnnn

SEQ ID NO: 26 - DNA, 61 bp, Sus scrofa
cccggtgcccggggcctctggcccttgtcgacgattctggatcagtcccaacaccacctgg

SEQ ID NO: 27 - DNA, 61 bp, Sus scrofa
cccggtgcccggggcccttgtcgacgatcagcccttctggatcagtcccaacaccacctgg

SEQ ID NO: 28 - DNA, 356 bp, Sus scrofa
tcagcgcttgaccttgcggccggctgaattgcgcccactgcggcgatagagagactgctggccgccgttgagcgggcagtacttgagtgtgtgagcctggtcaccggtggccccgcacaggggacacacatagtgtcgtaggatgggacacaccaccacgccctccggtgtcttcagctggtgcgaggagtacacgtggcgagattccccattgtgtttgcaaaagttgcacagggtggccagccccccgctggccccccgctctcccgggccctggtcctgctccagtgggggctcaggtcttggctcctcaggttgaagtagtccttccacatgtcaaagggtggcagctgcat

SEQ ID NO: 29 - DNA, 56 bp, Sus scrofa
ttggctccccggtgcccggggcctctggcccttgtcgacgattctggatcagtccc

SEQ ID NO: 30 - DNA, 56 bp, Sus scrofa; identical to SEQ ID NO: 29

SEQ ID NO: 31 - DNA, 49 bp, Sus scrofa
ttggctccccggtgcccggggcctctgtcgacgattctggatcagtccc

SEQ ID NO: 32 - DNA, 49 bp, Sus scrofa; identical to SEQ ID NO: 31

SEQ ID NO: 33 - DNA, 55 bp, Sus scrofa
ttggctcccggtgcccggggcctctggcccttgtcgacgattctggatcagtccc

SEQ ID NO: 34 - DNA, 54 bp, Sus scrofa
ttggctccccggtgcccggggcctctgcccttgtccacaattctggatcatccc

SEQ ID NO: 35 - DNA, 49 bp, Sus scrofa; identical to SEQ ID NO: 31

SEQ ID NO: 36 - DNA, 49 bp, Sus scrofa
ttggctccccggtgcccggtgcccttgtcgacgattctggatcagtccc

SEQ ID NO: 37 - DNA, 49 bp, Sus scrofa
ttggctccccggtgcccggggcccttgtcgacgattctggatcagtccc

SEQ ID NO: 38 - DNA, 54 bp, Sus scrofa
ttggctccccggtgcccggggcctctgccttgtcgacgattctggatcagtccc

SEQ ID NO: 39 - DNA, 49 bp, Sus scrofa; identical to SEQ ID NO: 31

SEQ ID NO: 40 - DNA, 50 bp, Sus scrofa
ttggctccccggtgcccggggccccttgtcgacgattctggatcagtccc

SEQ ID NO: 41 - DNA, 55 bp, Sus scrofa
ttggctccccggtgcccggggcctctgcccttgtcgtcaattctggatcagtccc

SEQ ID NO: 42 - DNA, 49 bp, Sus scrofa
ttggctccccggtgcccggggcctctgtcgacaattctggatcagtccc

SEQ ID NO: 43 - DNA, 9289 bp, Artificial Sequence
  Synthetic polynucleotide
gagggcctatttcccatgattccttcatatttgcatatacgatacaaggctgttagagagataattggaattaatttgactgtaaacacaaagatattagtacaaaatacgtgacgtagaaagtaataatttcttgggtagtttgcagttttaaaattatgttttaaaatggactatcatatgcttaccgtaacttgaaagtatttcgatttcttggctttatatatcttgtggaaaggacgaaacaccgggtcttcgagaagacctgttttagagctagaaatagcaagttaaaataaggctagtccgttatcaacttgaaaaagtggcaccgagtcggtgcttttttgttttagagctagaaatagcaagttaaaataaggctagtccgtttttagcgcgtgcgccaattctgcagacaaatggctctagaggtacccgttacataacttacggtaaatggcccgcctggctgaccgcccaacgacccccgcccattgacgtcaatagtaacgccaatagggactttccattgacgtcaatgggtggagtatttacggtaaactgcccacttggcagtacatcaagtgtatcatatgccaagtacgccccctattgacgtcaatgacggtaaatggcccgcctggcattgtgcccagtacatgaccttatgggactttcctacttggcagtacatctacgtattagtcatcgctattaccatggtcgaggtgagccccacgttctgcttcactctccccatctcccccccctccccacccccaattttgtatttatttattttttaattattttgtgcagcgatgggggcggggggggggggggggcgcgcgccaggcggggcggggcggggcgaggggcggggcggggcgaggcggagaggtgcggcggcagccaatcagagcggcgcgctccgaaagtttccttttatggcgaggcggcggcggcggcggccctataaaaagcgaagcgcgcggcgggcgggagtcgctgcgacgctgccttcgccccgtgccccgctccgccgccgcctcgcgccgcccgccccggctctgactgaccgcgttactcccacaggtgagcgggcgggacggcccttctcctccgggctgtaattagctgagcaagaggtaagggtttaagggatggttggttggtggggtattaatgtttaattacctggagcacctgcctgaaatcaatgacgataagatggccccaaagaagaagcggaaggtcggtatccacggagtcccagcagccgacaagaagtacagcatcggcctggacatcggcaccaactctgtgggctgggccgtgatcaccgacgagtacaaggtgcccagcaagaaattcaaggtgctgggcaacaccgaccggcacagcatcaagaagaacctgatcggagccctgctgttcgacagcggcgaaacagccgaggccacccggctgaagagaaccgccagaagaagatacaccagacggaagaaccggatctgctatctgcaagagatcttcagcaacgagatggccaaggtggacgacagcttcttccacagactggaagagtccttcctggtggaagaggataagaagcacgagcggcaccccatcttcggcaacatcgtggacgaggtggcctaccacgagaagtaccccaccatctaccacctgagaaagaaactggtggacagcaccgacaaggccgacctgcggctgatctatctggccctggcccacatgatcaagttccggggccacttcctgatcgagggcgacctgaaccccgacaacagcgacgtggacaagctgttcatccagctggtgcagacctacaaccagctgttcgaggaaaaccccatcaacgccagcggcgtggacgccaaggccatcctgtctgccagactgagcaagagcagacggctggaaaatctgatcgcccagctgcccggcgagaagaagaatggcctgttcggaaacctgattgccctgagcctgggcctgacccccaacttcaagagcaacttcgacctggccgaggatgccaaactgcagctgagcaaggacacctacgacgacgacctggacaacctgctggcccagatcggcgaccagtacgccgacctgtttctggccgccaagaacctgtccgacgccatcctgctgagcgacatcctgagagtgaacaccgagatcaccaaggcccccctgagcgcctctatgatcaagagatacgacgagcaccaccaggacctgaccctgctgaaagctctcgtgcggcagcagctgcctgagaagtacaaagagattttcttcgaccagagcaagaacggctacgccggctacattgacggcggagccagccaggaagagttctacaagttcatcaagcccatcctggaaaagatggacggcaccgaggaactgctcgtgaagctgaacagagaggacctgctgcggaagcagcggaccttcgacaacggcagcatcccccaccagatccacctgggagagctgcacgccattctgcggcggcaggaagatttttacccattcctgaaggacaaccgggaaaagatcgagaagatcctgaccttccgcatcccctactacgtgggccctctggccaggggaaacagcagattcgcctggatgaccagaaagagcgaggaaaccatcaccccctggaacttcgaggaagtggtggacaagggcgcttccgcccagagcttcatcgagcggatgaccaacttcgataagaacctgcccaacgagaaggtgctgcccaagcacagcctgctgtacgagtacttcaccgtgtataacgagctgaccaaagtgaaatacgtgaccgagggaatgagaaagcccgccttcctgagcggcgagcagaaaaaggccatcgtggacctgctgttcaagaccaaccggaaagtgaccgtgaagcagctgaaagaggactacttcaagaaaatcgagtgcttcgactccgtggaaatctccggcgtggaagatcggttcaacgcctccctgggcacataccacgatctgctgaaaattatcaaggacaaggacttcctggacaatgaggaaaacgaggacattctggaagatatcgtgctgaccctgacactgtttgaggacagagagatgatcgaggaacggctgaaaacctatgcccacctgttcgacgacaaagtgatgaagcagctgaagcggcggagatacaccggctggggcaggctgagccggaagctgatcaacggcatccgggacaagcagtccggcaagacaatcctggatttcctgaagtccgacggcttcgccaacagaaacttcatgcagctgatccacgacgacagcctgacctttaaagaggacatccagaaagcccaggtgtccggccagggcgatagcctgcacgagcacattgccaatctggccggcagccccgccattaagaagggcatcctgcagacagtgaaggtggtggacgagctcgtgaaagtgatgggccggcacaagcccgagaacatcgtgatcgaaatggccagagagaaccagaccacccagaagggacagaagaacagccgcgagagaatgaagcggatcgaagagggcatcaaagagctgggcagccagatcctgaaagaacaccccgtggaaaacacccagctgcagaacgagaagctgtacctgtactacctgcagaatgggcgggatatgtacgtggaccaggaactggacatcaaccggctgtccgactacgatgtggaccatatcgtgcctcagagctttctgaaggacgactccatcgacaacaaggtgctgaccagaagcgacaagaaccggggcaagagcgacaacgtgccctccgaagaggtcgtgaagaagatgaagaactactggcggcagctgctgaacgccaagctgattacccagagaaagttcgacaatctgaccaaggccgagagaggcggcctgagcgaactggataaggccggcttcatcaagagacagctggtggaaacccggcagatcacaaagcacgtggcacagatcctggactcccggatgaacactaagtacgacgagaatgacaagctgatccgggaagtgaaagtgatcaccctgaagtccaagctggtgtccgatttccggaaggatttccagttttacaaagtgcgcgagatcaacaactaccaccacgcccacgacgcctacctgaacgccgtcgtgggaaccgccctgatcaaaaagtaccctaagctggaaagcgagttcgtgtacggcgactacaaggtgtacgacgtgcggaagatgatcgccaagagcgagcaggaaatcggcaaggctaccgccaagtacttcttctacagcaacatcatgaactttttcaagaccgagattaccctggccaacggcgagatccggaagcggcctctgatcgagacaaacggcgaaaccggggagatcgtgtgggataagggccgggattttgccaccgtgcggaaagtgctgagcatgccccaagtgaatatcgtgaaaaagaccgaggtgcagacaggcggcttcagcaaagagtctatcctgcccaagaggaacagcgataagctgatcgccagaaagaaggactgggaccctaagaagtacggcggcttcgacagccccaccgtggcctattctgtgctggtggtggccaaagtggaaaagggcaagtccaagaaactgaagagtgtgaaagagctgctggggatcaccatcatggaaagaagcagcttcgagaagaatcccatcgactttctggaagccaagggctacaaagaagtgaaaaaggacctgatcatcaagctgcctaagtactccctgttcgagctggaactttttttcaggttggaccggtgccaccatggactataaggaccacgacggagactacaaggatcatgatattgattacaaagacgaacggccggaagagaatgctggcctctgccggcgaactgcagaagggaaacgaactggccctgccctccaaatatgtgaacttcctgtacctggccagccactatgagaagctgaagggctcccccgaggataatgagcagaaacagctgtttgtggaacagcacaagcactacctggacgagatcatcgagcagatcagcgagttctccaagagagtgatcctggccgacgctaatctggacaaagtgctgtccgcctacaacaagcaccgggataagcccatcagagagcaggccgagaatatcatccacctgtttaccctgaccaatctgggagcccctgccgccttcaagtactttgacaccaccatcgaccggaagaggtacaccagcaccaaagaggtgctggacgccaccctgatccaccagagcatcaccggcctgtacgagacacggatcgacctgtctcagctgggaggcgacaaaaggccggcggccacgaaaaaggccggccaggcaaaaaagaaaaaggaattcggcagtggagagggcagaggaagtctgctaacatgcggtgacgtcgaggagaatcctggcccagtgagcaagggcgaggagctgttcaccggggtggtgcccatcctggtcgagctggacggcgacgtaaacggccacaagttcagcgtgtccggcgagggcgagggcgatgccacctacggcaagctgaccctgaagttcatctgcaccaccggcaagctgcccgtgccctggcccaccctcgtgaccaccctgacctacggcgtgcagtgcttcagccgctaccccgaccacatgaagcagcacgacttcttcaagtccgccatgcccgaaggctacgtccaggagcgcaccatcttcttcaaggacgacggcaactacaagacccgcgccgaggtgaagttcgagggcgacaccctggtgaaccgcatcgagctgaagggcatcgacttcaaggaggacggcaacatcctggggcacaagctggagtacaactacaacagccacaacgtctatatcatggccgacaagcagaagaacggcatcaaggtgaacttcaagatccgccacaacatcgaggacggcagcgtgcagctcgccgaccactaccagcagaacacccccatcggcgacggccccgtgctgctgcccgacaaccactacctgagcacccagtccgccctgagcaaagaccccaacgagaagcgcgatcacatggtcctgctggagttcgtgaccgccgccgggatcactctcggcatggacgagctgtacaaggaattctaactagagctcgctgatcagcctcgactgtgccttctagttgccagccatctgttgtttgcccctcccccgtgccttccttgaccctggaaggtgccactcccactgtcctttcctaataaaatgaggaaattgcatcgcattgtctgagtaggtgtcattctattctggggggtggggtggggcaggacagcaagggggaggattgggaagagaatagcaggcatgctggggagcggccgcaggaacccctagtgatggagttggccactccctctctgcgcgctcgctcgctcactgaggccgggcgaccaaaggtcgcccgacgcccgggctttgcccgggcggcctcagtgagcgagcgagcgcgcagctgcctgcaggggcgcctgatgcggtattttctccttacgcatctgtgcggtatttcacaccgcatacgtcaaagcaaccatagtacgcgccctgtagcggcgcattaagcgcggcgggtgtggtggttacgcgcagcgtgaccgctacacttgccagcgccctagcgcccgctcctttcgctttcttcccttcctttctcgccacgttcgccggctttccccgtcaagctctaaatcgggggctccctttagggttccgatttagtgctttacggcacctcgaccccaaaaaacttgatttgggtgatggttcacgtagtgggccatcgccctgatagacggtttttcgccctttgacgttggagtccacgttctttaatagtggactcttgttccaaactggaacaacactcaaccctatctcgggctattcttttgatttataagggattttgccgatttcggcctattggttaaaaaatgagctgatttaacaaaaatttaacgcgaattttaacaaaatattaacgtttacaattttatggtgcactctcagtacaatctgctctgatgccgcatagttaagccagccccgacacccgccaacacccgctgacgcgccctgacgggcttgtctgctcccggcatccgcttacagacaagctgtgaccgtctccgggagctgcatgtgtcagaggttttcaccgtcatcaccgaaacgcgcgagacgaaagggcctcgtgatacgcctatttttataggttaatgtcatgataataatggtttcttagacgtcaggtggcacttttcggggaaatgtgcgcggaacccctatttgtttatttttctaaatacattcaaatatgtatccgctcatgagacaataaccctgataaatgcttcaataatattgaaaaaggaagagtatgagtattcaacatttccgtgtcgcccttattcccttttttgcggcattttgccttcctgtttttgctcacccagaaacgctggtgaaagtaaaagatgctgaagatcagttgggtgcacgagtgggttacatcgaactggatctcaacagcggtaagatccttgagagttttcgccccgaagaacgttttccaatgatgagcacttttaaagttctgctatgtggcgcggtattatcccgtattgacgccgggcaagagcaactcggtcgccgcatacactattctcagaatgacttggttgagtactcaccagtcacagaaaagcatcttacggatggcatgacagtaagagaattatgcagtgctgccataaccatgagtgataacactgcggccaacttacttctgacaacgatcggaggaccgaaggagctaaccgcttttttgcacaacatgggggatcatgtaactcgccttgatcgttgggaaccggagctgaatgaagccataccaaacgacgagcgtgacaccacgatgcctgtagcaatggcaacaacgttgcgcaaactattaactggcgaactacttactctagcttcccggcaacaattaatagactggatggaggcggataaagttgcaggaccacttctgcgctcggcccttccggctggctggtttattgctgataaatctggagccggtgagcgtggaagccgcggtatcattgcagcactggggccagatggtaagccctcccgtatcgtagttatctacacgacggggagtcaggcaactatggatgaacgaaatagacagatcgctgagataggtgcctcactgattaagcattggtaactgtcagaccaagtttactcatatatactttagattgatttaaaacttcatttttaatttaaaaggatctaggtgaagatcctttttgataatctcatgaccaaaatcccttaacgtgagttttcgttccactgagcgtcagaccccgtagaaaagatcaaaggatcttcttgagatcctttttttctgcgcgtaatctgctgcttgcaaacaaaaaaaccaccgctaccagcggtggtttgtttgccggatcaagagctaccaactctttttccgaaggtaactggcttcagcagagcgcagataccaaatactgtccttctagtgtagccgtagttaggccaccacttcaagaactctgtagcaccgcctacatacctcgctctgctaatcctgttaccagtggctgctgccagtggcgataagtcgtgtcttaccgggttggactcaagacgatagttaccggataaggcgcagcggtcgggctgaacggggggttcgtgcacacagcccagcttggagcgaacgacctacaccgaactgagatacctacagcgtgagctatgagaaagcgccacgcttcccgaagggagaaaggcggacaggtatccggtaagcggcagggtcggaacaggagagcgcacgagggagcttccagggggaaacgcctggtatctttatagtcctgtcgggtttcgccacctctgacttgagcgtcgatttttgtgatgctcgtcaggggggcggagcctatggaaaaacgccagcaacgcggcctttttacggttcctggccttttgctggccttttgctcacatgt

SEQ ID NO: 44 - DNA, 61 bp, Sus scrofa
ctcaggtcttggctccccggtgcccggggcctctggcccttgtcgacgattctggatcagt

SEQ ID NO: 45 - DNA, 60 bp, Sus scrofa
ctcaggtcttggctccccggtgcccggggcctctgcccttgtcgacgattctggatcagt

SEQ ID NO: 46 - DNA, 60 bp, Sus scrofa
ctcaggtcttggctccccggtgcccggtgcccgggcccttgtcgacgattctggatcagt

SEQ ID NO: 47 - DNA, 60 bp, Sus scrofa; identical to SEQ ID NO: 46

SEQ ID NO: 48 - DNA, 54 bp, Sus scrofa
  misc_feature (6)..(7): n is a, c, g, or t
atcagnncttggctccccggtgcccggggcctctggccacgattctggatcagt

SEQ ID NO: 49 - DNA, 54 bp, Sus scrofa
ctcaggtcttggctccccggtgcccggggcctctgtcgacgattctggatcagt

SEQ ID NO: 50 - DNA, 54 bp, Sus scrofa; identical to SEQ ID NO: 49

SEQ ID NO: 51 - DNA, 59 bp, Sus scrofa
ctcaggtcttggctccccggtgcccggggcctctggcccttgtcgacttctggatcagt

SEQ ID NO: 52 - DNA, 60 bp, Sus scrofa; identical to SEQ ID NO: 45

SEQ ID NO: 53 - DNA, 24 bp, Sus scrofa
gcaccagctgaagaccaccggagg

SEQ ID NO: 54 - DNA, 23 bp, Sus scrofa
gctggtgcgaggagtacacgtgg

SEQ ID NO: 55 - DNA, 65 bp, Sus scrofa
gaatctcgccacgtgtactcctcgcaccagctgaagacaccggagggcgtggtggtgtgtcccat

SEQ ID NO: 56 - DNA, 64 bp, Sus scrofa
gaatctcgccacgtgtactcctcgcaccagctgaagacaccggagggcgtggtggtgttcccat

SEQ ID NO: 57 - DNA, 65 bp, Sus scrofa; identical to SEQ ID NO: 55

SEQ ID NO: 58 - DNA, 64 bp, Sus scrofa; identical to SEQ ID NO: 56

SEQ ID NO: 59 - DNA, 65 bp, Sus scrofa; identical to SEQ ID NO: 55

SEQ ID NO: 60 - DNA, 65 bp, Sus scrofa; identical to SEQ ID NO: 55

SEQ ID NO: 61 - DNA, 65 bp, Sus scrofa; identical to SEQ ID NO: 55

SEQ ID NO: 62 - DNA, 1000 bp, Bovine
gaaggatgggggtgggggcgtttgcagacatgaagttttgttgaaaggacagaaaaactgaggcccagggagacgggtctttccagaggtcacagagcaccttgcaggccaagcaagcaccagagacaacaggaaagacccccttccacatctccatggggaattaaagtcagaaggaatcaaaggtgaggagtgggccctttaaatcctaagctccacctttgcttagaagggtctttgggaatataaaagggggtgcagttcctctctgctcctgaaaaccatcagctgctcctgtctgcgggcccccagcccacttctctccagccacccaccaccaacactcccccgggtgccatgcagctgccaccctttgacatgtggaaggactacttcaacctgagccaagtggtgctggcactgatccagagtcgggggcaagggttggagacccaagggactggggagccgagacccgggccccatgtggagcaggatcaggggcagggcggacgcggggctggcgggggcctggccaccctgtgcaacttttgcaaacacaatggagagtctcgccacgtgtactcctcacaccagctgaagaccccggagggcgtggtggtgtgtcccattctgcggcattatgtatgtcccctgtgcggggccaccggggaccaggcccacacactcaagtactgcccactcaacggaggacagcagtctctctaccgccgcagtgggcgcaactcagccggccgcaaggtcaagcgctgaagaccgtcaggtacccacccgctgcagccccaaccctccctggttcagccctcccaagcccctggactctccccatctatggactcgtcaggccctttggaatgtctgactctcagtacttgatccctgctggatcctggaacaacggaggcagtgggaagccaggccaactccgcggccccttagaactctcagctctccggactcttgtctgcgagtgtctgtg

SEQ ID NO: 63 - DNA, 417 bp, Bovine
atgcagctgccaccctttgacatgtggaaggactacttcaacctgagccaagtggtgctggcactgatccagagtcgggggcaagggttggagacccaagggactggggagccgagacccgggccccatgtggagcaggatcaggggcagggcggacgcggggctggcgggggcctggccaccctgtgcaacttttgcaaacacaatggagagtctcgccacgtgtactcctcacaccagctgaagaccccggagggcgtggtggtgtgtcccattctgcggcattatgtatgtcccctgtgcggggccaccggggaccaggcccacacactcaagtactgcccactcaacggaggacagcagtctctctaccgccgcagtgggcgcaactcagccggccgcaaggtcaagcgctga

SEQ ID NO: 64 - DNA, 20 bp, Bovine
agacgggtctttccagaggt

SEQ ID NO: 65 - DNA, 20 bp, Bovine
aagctccacctttgcttaga

SEQ ID NO: 66 - DNA, 21 bp, Bovine
ctttgcttagaagggtctttt

SEQ ID NO: 67 - DNA, 20 bp, Bovine
ggtctttgggaatataaaag

SEQ ID NO: 68 - DNA, 19 bp, Bovine
ggcaagggttggagaccca

SEQ ID NO: 69 - DNA, 20 bp, Bovine
gccgagacccgggccccatg

SEQ ID NO: 70 - DNA, 20 bp, Bovine
cccatgtggagcaggatcag

SEQ ID NO: 71 - DNA, 19 bp, Bovine
tccccatctctggactcgt

SEQ ID NO: 72 - DNA, 20 bp, Bovine
tctggactcgtccggccctt

SEQ ID NO: 73 - DNA, 20 bp, Bovine
tctcagtacttgatccctgc

SEQ ID NO: 74 - DNA, 20 bp, Bovine
acaagagtccggagagctga

SEQ ID NO: 75 - DNA, 54 bp, Sus scrofa
tgccatgcagctgccaccctttgacatgtggaaggactacttcaacctgagcca

SEQ ID NO: 76 - DNA, 18 bp, Sus scrofa
tgccatgcagctgccacc

SEQ ID NO: 77 - DNA, 18 bp, Sus scrofa
tggctcaggttgaagtag

SEQ ID NO: 78 - DNA, 52 bp, Sus scrofa
tttgacatgtggaaggactacttcaacctgagccaggtggtgttgggactga

SEQ ID NO: 79 - DNA, 18 bp, Sus scrofa
tttgacatgtggaaggac

SEQ ID NO: 80 - DNA, 18 bp, Sus scrofa
tcagtcccaacaccacct

SEQ ID NO: 81 - DNA, 53 bp, Sus scrofa
tcaacctgagccaggtggtgttgggactgatccagaatcgtcgacaagggcca

SEQ ID NO: 82 - DNA, 18 bp, Sus scrofa
tcaacctgagccaggtgg

SEQ ID NO: 83 - DNA, 16 bp, Sus scrofa
gcccttgtcgacgatt

SEQ ID NO: 84 - DNA, 19 bp, Sus scrofa
gcgggcagtacttgagtgt

SEQ ID NO: 85 - DNA, 20 bp, Sus scrofa
ccagaaaaccttctgctgct

SEQ ID NO: 86 - DNA, 26 bp, Sus scrofa
ccagaatcgtcgacaagggccagagg

SEQ ID NO: 87 - DNA, 26 bp, Sus scrofa
ggtcttagcagctgttcccggtctcc

SEQ ID NO: 88 - DNA, 24 bp, Bovine
caccggtctttgggaatataaaag

SEQ ID NO: 89 - DNA, 24 bp, Bovine
aaaccttttatattcccaaagacc

SEQ ID NO: 90 - DNA, 23 bp, Bovine
caccgtctttgggaatataaaag

SEQ ID NO: 91 - DNA, 23 bp, Bovine
aaaccttttatattcccaaagac

SEQ ID NO: 92 - DNA, 25 bp, Bovine
caccgctttgcttagaagggtcttt

SEQ ID NO: 93 - DNA, 25 bp, Bovine
aaacaaagacccttctaagcaaagc

SEQ ID NO: 94 - DNA, 23 bp, Bovine
caccgttgcttagaagggtcttt

SEQ ID NO: 95 - DNA, 22 bp, Bovine
aacaaagacccttctaagcaac

SEQ ID NO: 96 - DNA, 25 bp, Bovine
caccgagctccacctttgcttagaa

SEQ ID NO: 97 - DNA, 25 bp, Bovine
aaacttctaagcaaaggtggagctc

SEQ ID NO: 98 - DNA, 23 bp, Bovine
caccgctccacctttgcttagaa

SEQ ID NO: 99 - DNA, 23 bp, Bovine
aaacttctaagcaaaggtggagc

SEQ ID NO: 100 - DNA, 24 bp, Bovine
caccggcaagggttggagacccaa

SEQ ID NO: 101 - DNA, 24 bp, Bovine
aaacttgggtctccaacccttgcc

SEQ ID NO: 102 - DNA, 23 bp, Bovine
caccgcaagggttggagacccaa

SEQ ID NO: 103 - DNA, 23 bp, Bovine
aaacttgggtctccaacccttgc

SEQ ID NO: 104 - DNA, 24 bp, Bovine
caccgccgagacccgggccccatg

SEQ ID NO: 105 - DNA, 24 bp, Bovine
aaaccatggggcccgggtctcggc

SEQ ID NO: 106 - DNA, 21 bp, Bovine
caccgagacccgggccccatg

SEQ ID NO: 107 - DNA, 21 bp, Bovine
aaaccatggggcccgggtctc

SEQ ID NO: 108 - DNA, 25 bp, Bovine
caccgcccatgtggagcaggatcag

SEQ ID NO: 109 - DNA, 25 bp, Bovine
aaacctgatcctgctccacatgggc

SEQ ID NO: 110 - DNA, 23 bp, Bovine
caccgcatgtggagcaggatcag

SEQ ID NO: 111 - DNA, 23 bp, Bovine
aaacctgatcctgctccacatgc

SEQ ID NO: 112 - DNA, 25 bp, Bovine
caccgtccccatctctggactcgtc

SEQ ID NO: 113 - DNA, 25 bp, Bovine
aaacgacgagtccagagatggggac

SEQ ID NO: 114 - DNA, 23 bp, Bovine
caccgcccatctctggactcgtc

SEQ ID NO: 115 - DNA, 23 bp, Bovine
aaacgacgagtccagagatgggc

SEQ ID NO: 116 - DNA, 25 bp, Bovine
caccgtctggactcgtccggccctt

SEQ ID NO: 117 - DNA, 201 bp, Bovine
tgggccctttaaatcctaagctccacctttgcttagaagggtctttgggaatataaaagggggtgcagttcctgagccaagtggtgctggcactgatccagagtcgggggcaagggttggagacccaagggactggggagccgagacccggccccatgtggagcaggatcaggggcagggcggacgcggggccggcggggg

SEQ ID NO: 118 - DNA, 132 bp, Bovine
tgggccctttaaatcctaagctccacctttgcttagaagggtctttgggaatataacaagggactggggagccgagacccggccccatgtggagcaggatcaggggcagggcggacgcggggccggcggggg

SEQ ID NO: 119 - DNA, 132 bp, Bovine; identical to SEQ ID NO: 118

SEQ ID NO: 120 - DNA, 119 bp, Bovine
tgggccctttaaatcctaagctccacctttgcttagaagggtctttgggactggggagccgagacccggccccatgtggagcaggatcaggggcagggcggacgcggggccggcggggg

SEQ ID NO: 121 - DNA, 119 bp, Bovine; identical to SEQ ID NO: 120

SEQ ID NO: 122 - DNA, 112 bp, Bovine
tgggccctttaaatcctaagctccacctttgcttagaagggtctttgggagccgagacccggccccatgtggagcaggatcaggggcagggcggacgcggggccggcggggg

SEQ ID NO: 123 - DNA, 201 bp, Bovine; identical to SEQ ID NO: 117

SEQ ID NO: 124 - DNA, 129 bp, Bovine
tgggccctttaaatcctaagctccacctttgcttagaagggtctttgggggtgcagttcctgagccaagtggtgctggcactgatccagagtcgggggcaagggttggagacccaagggactggggagc

SEQ ID NO: 125 - DNA, 103 bp, Bovine
tgggccctttaaatcctaagctccacctttgcttagaagggtctttgggaatataacatgtggagcaggatcaggggcagggcggacgcggggccggcggggg

SEQ ID NO: 126 - DNA, 104 bp, Bovine
tgggccctttaaatcctaagctccacctttgcttagaagggtctttgggaatataaacatgtggagcaggatcaggggcagggcggacgcggggccggcggggg

SEQ ID NO: 127 - DNA, 106 bp, Bovine
tgggccctttaaatcctaagctccacctttgcttagaagggtctttgggagtgcagttccatgtggagcaggatcaggggcagggcggacgcggggccggcggggg

SEQ ID NO: 128 - DNA, 103 bp, Bovine; identical to SEQ ID NO: 125

SEQ ID NO: 129 - DNA, 201 bp, Bovine; identical to SEQ ID NO: 117

SEQ ID NO: 130 - DNA, 48 bp, Bovine
tgggccctttaaatcctaagctccacctttgcttagaagggtctaagg

SEQ ID NO: 131 - DNA, 89 bp, Bovine
tgggccctttaaatcctaagctccacctttgcttagaagggtctttgggaatataatcaggggcagggcggacgcggggccggcggggg

SEQ ID NO: 132 - DNA, 88 bp, Bovine
tgggccctttaaatcctaagctccacctttgcttagaagggtctttgggaatataacaggggcagggcggacgcggggccggcggggg

SEQ ID NO: 133 - DNA, 45 bp, Bovine
tgggccctttaaatcctaagctccacctttgctggccgggggggg

SEQ ID NO: 134 - DNA, 62 bp, Bovine
tgggccctttaaatcctaagctccacctttgcttagaagggcggacgcggggccggcggggg

SEQ ID NO: 135 - DNA, 200 bp, Bovine
tgggccctttaaatcctaagctccacctttgcttagaagggtctttgggaatataaaagggggtgcagttcctgagccaagtggtgctggcactgatccagagtcgggggcaagggttggagacccaagggactggggagccgagacccggccccatgtggagcaggatcaggggcagggcggacgcggggccggcgggg

SEQ ID NO: 136 - DNA, 132 bp, Bovine; identical to SEQ ID NO: 118

SEQ ID NO: 137 - DNA, 132 bp, Bovine; identical to SEQ ID NO: 118

SEQ ID NO: 138 - DNA, 132 bp, Bovine; identical to SEQ ID NO: 118

SEQ ID NO: 139 - DNA, 132 bp, Bovine; identical to SEQ ID NO: 118

SEQ ID NO: 140 - DNA, 132 bp, Bovine; identical to SEQ ID NO: 118

SEQ ID NO: 141 - DNA, 201 bp, Bovine; identical to SEQ ID NO: 117

SEQ ID NO: 142 - DNA, 98 bp, Bovine
tgggccctttaaatcctaagctccacctttgcttagaagggtctttgggaatatgtggagcaggatcaggggcagggcggacgcggggccggcggggg

SEQ ID NO: 143 - DNA, 103 bp, Bovine; identical to SEQ ID NO: 125

SEQ ID NO: 144 - DNA, 89 bp, Bovine
tgggccctttaaatcctaagctccacctttgcttagaagggtctttgggaatatgatcaggggcagggcggacgcggggccggcggggg

SEQ ID NO: 145 - DNA, 89 bp, Bovine
tgggccctttaaatcctaagctccacctttgcttagaagggtctttgggagcaggatcaggggcagggcggacgcggggccggcggggg

SEQ ID NO: 146 - DNA, 103 bp, Bovine; identical to SEQ ID NO: 125

SEQ ID NO: 147 - DNA, 201 bp, Bovine; identical to SEQ ID NO: 117

SEQ ID NO: 148 - DNA, 68 bp, Bovine
tgggccctttaaatcctaagctccacctttgcttctcaggggcagggcggacgcggggccggcggggg

SEQ ID NO: 149 - DNA, 70 bp, Bovine
tgggccctttaaatcctaagctccacctttgcttagaagggtctttgggcggacgcggggccggcggggg

SEQ ID NO: 150 - DNA, 88 bp, Bovine
gggccctttaaatcctaagctccacctttgcttagaagggtctttgggaatataatcaggggcagggcggacgcggggccggcggggg

SEQ ID NO: 151 - DNA, 67 bp, Bovine
tgggccctttaaatcctaagctccacctttgcttagaagggcagggcggacgcggggccggcggggg

SEQ ID NO: 152 - DNA, 125 bp, Bovine
tgggccctttaaatcctaagctccacctttgcttagaagtggtgctggcactgatccagagtcgggggcaagggttggagacccaagggactggggagccgagacccggccccatgtggagcagg

SEQ ID NO: 153 - DNA, 25 bp, Bovine
aaacaagggccggacgagtccagac

SEQ ID NO: 154 - DNA, 21 bp, Bovine
caccggactcgtccggccctt

SEQ ID NO: 155 - DNA, 21 bp, Bovine
aaacaagggccggacgagtcc

SEQ ID NO: 156 - DNA, 25 bp, Bovine
caccgtctcagtacttgatccctgc

SEQ ID NO: 157 - DNA, 25 bp, Bovine
aaacgcagggatcaagtactgagac

SEQ ID NO: 158 - DNA, 23 bp, Bovine
caccgtcagtacttgatccctgc

SEQ ID NO: 159 - DNA, 23 bp, Bovine
aaacgcagggatcaagtactgac

SEQ ID NO: 160 - DNA, 22 bp, Sus scrofa
gatcagtcccaacaccacctgg

SEQ ID NO: 161 - DNA, 22 bp, Sus scrofa
ccaggtggtgttgggactgatc

SEQ ID NO: 162 - DNA, 23 bp, Sus scrofa
gaatcgtcgacaagggccagagg

SEQ ID NO: 163 - DNA, 42 bp, Sus scrofa
ctacttcaacctgagccaggtggtgttgggactgatccagaa

SEQ ID NO: 164 - DNA, 37 bp, Sus scrofa
ctacttcaacctgagccaggttgggactgatccagaa

SEQ ID NO: 165 - DNA, 39 bp, Sus scrofa
ctacttcaacctgagccaggtgttgggactgatccagaa

SEQ ID NO: 166 - DNA, 39 bp, Sus scrofa
ctacttcaacctgagccagggactgggactgatccagaa

SEQ ID NO: 167 - DNA, 43 bp, Sus scrofa
ctacttcaacctgagccaggtgggtgttgggactgatccagaa

SEQ ID NO: 168 - DNA, 41 bp, Sus scrofa
ctacttcaacctgagccaggtgtgttgggactgatccagaa

SEQ ID NO: 169 - DNA, 37 bp, Sus scrofa
ctacttcaacctgagccaggttgggaccgatccagaa

SEQ ID NO: 170 - DNA, 39 bp, Sus scrofa; identical to SEQ ID NO: 165

SEQ ID NO: 171 - DNA, 39 bp, Sus scrofa; identical to SEQ ID NO: 165

SEQ ID NO: 172 - DNA, 32 bp, Sus scrofa
ctacttcaacctgagccaggactgatccagaa

SEQ ID NO: 173 - DNA, 39 bp, Sus scrofa; identical to SEQ ID NO: 165

SEQ ID NO: 174 - DNA, 39 bp, Sus scrofa; identical to SEQ ID NO: 165

SEQ ID NO: 175 - DNA, 37 bp, Sus scrofa; identical to SEQ ID NO: 164

SEQ ID NO: 176 - DNA, 39 bp, Sus scrofa
ctacttcaacctgagtcaggtgttgggactgatccagaa

SEQ ID NO: 177 - DNA, 45 bp, Sus scrofa
ctacttcaacctaagccaggttgaagtgttgggactgatccagaa

SEQ ID NO: 178 - DNA, 39 bp, Sus scrofa; identical to SEQ ID NO: 165

SEQ ID NO: 179 - DNA, 41 bp, Sus scrofa; identical to SEQ ID NO: 168

SEQ ID NO: 180 - DNA, 38 bp, Sus scrofa
ctacctcaacctgagccaggggtgggactgatccagaa

SEQ ID NO: 181 - DNA, 41 bp, Sus scrofa
ctacttcaacctgagcctggtgtgttgggactgatccagaa

SEQ ID NO: 182 - DNA, 39 bp, Sus scrofa; identical to SEQ ID NO: 165

SEQ ID NO: 183 - DNA, 39 bp, Sus scrofa; identical to SEQ ID NO: 165

SEQ ID NO: 184 - DNA, 38 bp, Sus scrofa
ctacttcaacctgagccaggtctgggactgatccagaa

SEQ ID NO: 185 - DNA, 16 bp, Sus scrofa
tgggactgatccagaa

SEQ ID NO: 186 - DNA, 45 bp, Sus scrofa
ctacttcaacctgagccaggttgaagtgttgggactgatccagaa

SEQ ID NO: 187 - DNA, 45 bp, Sus scrofa; identical to SEQ ID NO: 186

SEQ ID NO: 188 - DNA, 39 bp, Sus scrofa; identical to SEQ ID NO: 165

SEQ ID NO: 189 - DNA, 39 bp, Sus scrofa; identical to SEQ ID NO: 165

SEQ ID NO: 190 - DNA, 37 bp, Sus scrofa; identical to SEQ ID NO: 164

SEQ ID NO: 191 - DNA, 37 bp, Sus scrofa; identical to SEQ ID NO: 164

SEQ ID NO: 192 - DNA, 41 bp, Sus scrofa
ctacttcaacctgagccaggtgtgttgggactgatcaataa

SEQ ID NO: 193 - DNA, 38 bp, Sus scrofa
ctacttcaacctgagccagtgttgggactgatccagaa

SEQ ID NO: 194 - DNA, 39 bp, Sus scrofa; identical to SEQ ID NO: 165

SEQ ID NO: 195 - DNA, 42 bp, Sus scrofa
ctacttcaacctgagccaggcggggttgggactgatccagaa

SEQ ID NO: 196 - DNA, 39 bp, Sus scrofa; identical to SEQ ID NO: 165

SEQ ID NO: 197 - DNA, 37 bp, Sus scrofa; identical to SEQ ID NO: 164

SEQ ID NO: 198 - DNA, 41 bp, Sus scrofa; identical to SEQ ID NO: 168

SEQ ID NO: 199 - DNA, 21 bp, Sus scrofa
ctacttcaacctgagccagaa

SEQ ID NO: 200 - DNA, 51 bp, Sus scrofa
atccagaatcgtcgacaagggccagaggccccgggcaccggggagccaaga

SEQ ID NO: 201 - DNA, 44 bp, Sus scrofa
atccagaatcgtcgacaagggccccgggcaccggggagccaaga

SEQ ID NO: 202 - DNA, 44 bp, Sus scrofa; identical to SEQ ID NO: 201

SEQ ID NO: 203 - DNA, 50 bp, Sus scrofa
atccagaatcgtcgacgacgcgagaagccccgggcaccggggagccaaga

SEQ ID NO: 204 - DNA, 40 bp, Sus scrofa
atccagaatcgtcgaggccccgggcaccggggagccaaga